European Patent Specification EP 3 452 602 B1, published April 2, 2025. Title: Amylopectin potato starch with improved stability against retrogradation and  improved freeze and thaw stability. Applicant: Lyckeby Starch AB. The sequence listing filed with the application follows.

SEQUENCE LISTING (44 sequences)

SEQ ID NO: 1 - DNA, 20 bp, Solanum tuberosum
gatattagaatcacataggg

SEQ ID NO: 2 - DNA, 20 bp, Solanum tuberosum
tgttgacaagggtgttgaat

SEQ ID NO: 3 - DNA, 20 bp, Solanum tuberosum
gctaccattgtttgtggaaa

SEQ ID NO: 4 - DNA, 20 bp, Solanum tuberosum
gacaagaagatccctttgat

SEQ ID NO: 5 - DNA, 20 bp, Solanum tuberosum
gtgctaaaaggggtaagttg

SEQ ID NO: 6 - DNA, 20 bp, Solanum tuberosum
ggggtgccctttcatcggcc

SEQ ID NO: 7 - DNA, 20 bp, Solanum tuberosum
gctccagtagagagcaaatg

SEQ ID NO: 8 - DNA, 20 bp, Solanum tuberosum
gaacatctgaaccaaatttc

SEQ ID NO: 9 - DNA, 20 bp, Solanum tuberosum
gaggtggcaatggacccagg

SEQ ID NO: 10 - DNA, 20 bp, Solanum tuberosum
ggaaactaatgccagtagca

SEQ ID NO: 11 - DNA, 29 bp, Artificial sequence
  primer
cctcttctcaatcttcctgatgaattcag

SEQ ID NO: 12 - DNA, 29 bp, Artificial sequence
  primer
agagcctcctttagtaaaggttttgcgtc

SEQ ID NO: 13 - DNA, 22 bp, Artificial sequence
  primer
tgcttcacaatccctaattctc

SEQ ID NO: 14 - DNA, 22 bp, Artificial sequence
  primer
atccaaaagtgtctcttgactg

SEQ ID NO: 15 - DNA, 23 bp, Artificial sequence
  primer
gcttagagaagcggctatgcgtg

SEQ ID NO: 16 - DNA, 27 bp, Artificial sequence
  primer
tccatcatatatgcatccaatggaacc

SEQ ID NO: 17 - DNA, 20 bp, Artificial sequence
  primer
actggatgaaggctgggata

SEQ ID NO: 18 - DNA, 20 bp, Artificial sequence
  primer
atttgtcagtcgctgggttc

SEQ ID NO: 19 - DNA, 21 bp, Artificial sequence
  primer
aggaaccatactctgactcac

SEQ ID NO: 20 - DNA, 19 bp, Artificial sequence
  primer
ttttgctccaaggaccaac

SEQ ID NO: 21 - DNA, 21 bp, Artificial sequence
  primer
tctctatacaggtcatggacg

SEQ ID NO: 22 - DNA, 22 bp, Artificial sequence
  primer
gcagcaacaagaatatctgaac

SEQ ID NO: 23 - DNA, 19 bp, Artificial sequence
  primer
tggaaatcagttccacccc

SEQ ID NO: 24 - DNA, 22 bp, Artificial sequence
  primer
catggctaaaacctttttgctc

SEQ ID NO: 25 - DNA, 21 bp, Artificial sequence
  primer
cgataaaaatacaccgcctgc

SEQ ID NO: 26 - DNA, 19 bp, Artificial sequence
  primer
tctggagggacattcaacg

SEQ ID NO: 27 - DNA, 20 bp, Artificial sequence
  primer
atccaagctggaagcagtgt

SEQ ID NO: 28 - DNA, 20 bp, Artificial sequence
  primer
gacatgggtgccattttcag

SEQ ID NO: 29 - DNA, 22 bp, Artificial sequence
  primer
tgatgacaaggatgctgtaaag

SEQ ID NO: 30 - DNA, 21 bp, Artificial sequence
  primer
tcaacatccacctgcaatatc

SEQ ID NO: 31 - DNA, 38 bp, Solanum tuberosum
gggatattagaatcacatagggtggttacagtgagccc

SEQ ID NO: 32 - DNA, 42 bp, Solanum tuberosum
ttgtctctgctgttgacaagggtgttgaattggacagtgtcc

SEQ ID NO: 33 - DNA, 44 bp, Solanum tuberosum
ctggatgctcagctaccattgtttgtaaagggaatgaacttgat

SEQ ID NO: 34 - DNA, 38 bp, Solanum tuberosum
cctgttgacaagaagatccctttgattggcttcatcgg

SEQ ID NO: 35 - DNA, 38 bp, Solanum tuberosum
ttttgggcctaagtgctaaaaggggtaagttggggtgg

SEQ ID NO: 36 - DNA, 32 bp, Solanum tuberosum
gggggtgccctttcatcggccaggtccctttt

SEQ ID NO: 37 - DNA, 38 bp, Solanum tuberosum
cagcgattaaatgaacatctgaaccaaatttcaggttt

SEQ ID NO: 38 - DNA, 38 bp, Solanum tuberosum
ggcaacattttctgaggtggcaatggacccaggcggtg

SEQ ID NO: 39 - DNA, 37 bp, Artificial sequence
  primer
taatacgactcactatagacaagaagatccctttgat

SEQ ID NO: 40 - DNA, 34 bp, Artificial sequence
  primer
ttctagctctaaaacatcaaagggatcttcttgt

SEQ ID NO: 41 - DNA, 37 bp, Artificial sequence
  primer
taatacgactcactatagaggtggcaatggacccagg

SEQ ID NO: 42 - DNA, 34 bp, Artificial sequence
  primer
ttctagctctaaaaccctgggtccattgccacct

SEQ ID NO: 43 - DNA, 37 bp, Artificial sequence
  primer
taatacgactcactatagctccagtagagagcaaatg

SEQ ID NO: 44 - DNA, 34 bp, Artificial sequence
  primer
ttctagctctaaaaccatttgctctctactggag